European Patent Application EP 4 520 837 A1, published March 12, 2025. Title: Method and kit for the enzymatic degradation of polythiourethanes. Applicant: ESSILOR INTERNATIONAL. Application EP. The sequence listing filed with the application follows.

SEQUENCE LISTING (7 sequences)

SEQ ID NO: 1 - protein, 462 aa, Candida antarctica
MRVSLRSITSLLAAATAAVLAAPATETLDRRAALPNPYDDPFYTTPSNIGTFAKGQVIQSRKVPTDIGNANNAASFQLQYRTTNTQNEAVADVATVWIPAKPASPPKIFSYQVYEDATALDCAPSYSYLTGLDQPNKVTAVLDTPIIIGWALQQGYYVVSSDHEGFKAAFIAGYEEGMAILDGIRALKNYQNLPSDSKVALEGYSGGAHATVWATSLADSYAPELNIVGASHGGTPVSAKDTFTFLNGGPFAGFALAGVSGLSLAHPDMESFIEARLNAKGQQTLKQIRGRGFCLPQVVLTYPFLNVFSLVNDTNLLNEAPIAGILKQETVVQAEASYTVSVPKFPRFIWHAIPDEIVPYQPAATYVKEQCAKGANINFSPYPIAEHLTAEIFGLVPSLWFIKQAFDGTTPKVICGTPIPAIAGITTPSADQVLGSDLANQLRSLNGKQSAFGKPFGPITPP

SEQ ID NO: 2 - protein, 450 aa, Sus scrofa
SEVCFPRLGCFSDDAPWAGIVQRPLKILPWSPKDVDTRFLLYTNQNQNNYQELVADPSTITNSNFRMDRKTRFIIHGFIDKGEEDWLSNICKNLFKVESVNCICVDWKGGSRTGYTQASQNIRIVGAEVAYFVEVLKSSLGYSPSNVHVIGHSLGSHAAGEAGRRTNGTIERITGLDPAEPCFQGTPELVRLDPSDAKFVDVIHTDAAPIIPNLGFGMSQTVGHLDFFPNGGKQMPGCQKNILSQIVDIDGIWEGTRDFVACNHLRSYKYYADSILNPDGFAGFPCDSYNVFTANKCFPCPSEGCPQMGHYADRFPGKTNGVSQVFYLNTGDASNFARWRYKVSVTLSGKKVTGHILVSLFGNEGNSRQYEIYKGTLQPDNTHSDEFDSDVEVGDLQKVKFIWYNNNVINPTLPRVGASKITVERNDGKVYDFCSQETVREEVLLTLNPC

SEQ ID NO: 3 - protein, 565 aa, Sus scrofa
MWLLPLVLTSLASSATWAGQPASPPVVDTAQGRVLGKYVSLEGLAQPVAVFLGVPFAKPPLGSLRFAPPQPAEPWSFVKNTTSYPPMCCQDPVVEQMTSDLFTNGKERLTLEFSEDCLYLNIYTPADLTKRGRLPVMVWIHGGGLVLGGAPMYDGVVLAAHENVVVVAIQYRLGIWGFFSTGDEHSRGNWGHLDQVAALHWVQENIANFGGDPGSVTIFGESAGGESVSVLVLSPLAKNLFHAISESGVALTVALVRKDMKAAAKQIAVLAGCKTTTSAVFVHCLRQKSEDELLDLTLKMKFLTLDFHGDQRESHPFLPTVVDGVLLPKMPEEILAEKDFNTVPYIVGINKQEFGWLLPTMMGFPLSEGKLDQKTATSLLWKSYPIANIPEELTPVATDKYLGGTDDPVKKKDLFLDLMGDVVFGVPSVTVARQHRDAGAPTYMYEFQYRPSFSSDKKPKTVIGDHGDEIFSVFGFPLLKGDAPEEEVSLSKTVMKFWANFARSGNPNGEGLPHWPMYDQEEGYLQIGVNTQAAKRLKGEEVAFWNDLLSKEAAKKPPKIKHAEL

SEQ ID NO: 4 - protein, 482 aa, unidentified
MTELTVQTRCGALKGTAGHGVRTWKSIPYAKPPVGELRFKAPEPPVPWDGVKNADSFGPVCPQPADLLSMSFSGDVPPQSEDCLYLNVFAPDSEGGKRPVMVWIHGGAFFLGAGSEPTYDASALAADGDVIVVTLNYRLGPFGFLHLFSIDDTYPGNIGMLDQIAALRWVKDNISAFGGDPDNVTVFGESAGGMSIASLMAMPDAKGLFHKAILESGASQTMTADVAKEITTAFIQEAGTDQLQELSVNDILKTADKLRNTIDQSIFHLLFQPAIDPATLPAEPAKAIADGAAEGIPMIIGTNRDEAYLFFTPDTDIHSEKKQQEYLLYHLGENSAKLAADLYPHSLTGQIDMMTDLKFWRPAVAFAQEQSQYAPVWMYRFDWHGETPPFHKAVHALELPFVFGNFDSLKKTLKEPLSEDVKQLSKLIQSAWIAFAKTGKPDTDQLHWPQYETGSRETIIFNTSVSTESDPDSAKRRILFQA

SEQ ID NO: 5 - protein, 293 aa, unidentified
MSASSLKFPIVLVHGLLGFDKIGGIYPYFYGIKEALEKAGAKVYIATLSALNSNELRGEQLLEFVRKVQAETGAAKVNLIGHSQGPLACRYVAATHPELIASVTSVNGVNHGSEVADLVRLALTPGRLPESIANAAMSAFGQLLSALAGSPRLPQSGIEALEALTSEGVAAFNKKYPQGLPAEWGGEGKELVNGVYYYSWSGIIDYNPLHQGANNLDPLHVAMLAFSILFTNERFQNDGLVGRYSSHLGKVIGSDYSMDHVDAINQLAGVVANNTDPVQLFVEHVARLKSKGL

SEQ ID NO: 6 - protein, 377 aa, unidentified
MEHGNRRGPGRACAHQDTVTLKAGTRRSTSAIARTAAGTAAAIAAAIAMAWPASATASSDYAKTRYPIVLVHGLTGAAKMGGVIDYWYGIPEVLRANGATVYVSTVPSFNSDEERALALQAYVRAVKLETGADKVNLIGHSQGGPTSRMLAAMSPQDVASVTTIGSPHRGSQLADVVLDVINGISSIPLAGPALVNVIQGVTNLLGWFNGLFNGQALNQDAIASARTLTSQGATEQNARLNATLAPGSQSALGPDCDTPGAVAEQRQGRDASGKLVTYTQAAYSWTGRGGPINLLRSNLLDPSTAAMAAAAGVMGMKGAGPNDGMVSVCSAKWGRVLSTDYYWNHLDEINQMLGMYQDVDPRTVILNHANRLRNDQL

SEQ ID NO: 7 - protein, 299 aa, unidentified
MKKLVALLIVGLFVSISLTGLGLAGGTAPYKCDTRYPVVLAHGMGASTKILGIVDYWYGIEDALKAEGASVYFTSVNAMGSTVDKAADFKQQFMEILAVTGAPKANIIGHSHGTLYTRYAISNLGLAPYVASYTSLAGPHRGSAVASLIMYDLPDWLLAAGGDVLNFVYTFIFGDTNPDSLQNALDLCPDYMVNTFNPNTPNIPGIYYQSWAAKAKTSCPSVILEPTWLIMLIEEGANDGLVSVESAKWGNFRGVEDAAWYSAGCDHLNIVGQLFGVTPGFDAPQFFVDIVEDLKGRGY